European Patent Application EP 4 656 728 A1, published December 3, 2025. Title: METHOD FOR DELAYING SENESCENCE OF HUMAN MESENCHYMAL STEM CELLS AND APPLICATION THEREOF. Applicant: Affiliated Hospital of Zunyi Medical University. Application EP. The sequence listing filed with the application follows.

SEQUENCE LISTING (1 sequence)

SEQ ID NO: 1 - DNA, 2706 bp, synthetic construct
  source 1..2706: mol_type = other DNA
atggaggcaaatcagtgccccctggttgtggaaccatcttacccagacctggtcatcaatgtaggagaagtgactcttggagaagaaaacagaaaaaagctgcagaaaattcagagagaccaagagaaggagagagttatgcgggctgcatgtgctttattaaactcaggaggaggagtgattcgaatggccaagaaggttgagcatcccgtggagatgggactggatttagaacagtctttgagagagcttattcagtcttcagatctgcaggctttctttgagaccaagcaacaaggaaggtgtttttacatttttgttaaatcttggagcagtggccctttccctgaagatcgctctgtcaagccccgcctttgcagcctcagttcttcattataccgtagatctgagacctctgtgcgttccatggactcaagagaggcattctgtttcctgaagaccaaaaggaagccaaaaatcttggaagaaggaccttttcacaaaattcacaagggtgtataccaagagctccctaactcggatcctgctgacccaaactcggatcctgctgacctaattttccaaaaagactatcttgaatatggtgaaatcctgccttttcctgagtctcagttagtagagtttaaacagttctctacaaaacacttccaagaatatgtaaaaaggacaattccagaatacgtccctgcatttgcaaacactggaggaggctatctttttattggagtggatgataagagtagggaagtcctgggatgtgcaaaagaaaatgttgaccctgactctttgagaaggaaaatagaacaagccatatacaaactaccttgtgttcatttttgccaaccccaacgcccgataaccttcacactcaaaattgtgaatgtgttaaaaaggggagagctctatggctatgcttgcatgatcagagtaaatcccttctgctgtgcagtgttctcagaagctcccaattcatggatagtggaggacaagtacgtctgcagcctgacaaccgagaaatgggtaggcatgatgacagacacagatccagatcttctacagttgtctgaagattttgaatgtcagctgagtctatctagtgggcctccccttagcagaccagtgtactccaagaaaggcctggaacataaaaaggaactccagcaacttttattttcagtcccaccaggatatttgcgatatactccagagtcactctggagggacctgatctcagagcacagaggactagaggagttaataaataagcaaatgcaacctttctttcggggaattttgatcttctctagaagttgggctgtggacctgaacttgcaggagaagccaggagtcatctgtgatgctctgctgatagcacagaacagcacccccattctctacaccattctcagggagcaagatgcagagggccaggactactgcactcgcaccgcctttactttgaagcagaagctagtgaacatggggggctacaccgggaaggtgtgtgtcagggccaaggtcctctgcctgagtcctgagagcagcgcagaggccttggaggctgcagtgtctccgatggattaccctgcgtcctatagccttgcaggcacccagcacatggaagccctgctgcagtccctcgtgattgtcttactcggcttcaggtctctcttgagtgaccagctcggctgtgaggttttaaatctgctcacagcccagcagtatgagatattctccagaagcctccgcaagaacagagagttgtttgtccacggcttacctggctcagggaagaccatcatggccatgaagatcatggagaagatcaggaatgtgtttcactgtgaggcacacagaattctctacgtttgtgaaaaccagcctctgaggaactttatcagtgatagaaatatctgccgagcagagacccggaaaactttcctaagagaaaactttgaacacattcaacacatcgtcattgacgaagctcagaatttccgtactgaagatggggactggtatgggaaggcaaaaagcatcactcggagagcaaagggtggcccaggaattctctggatctttctggattactttcagaccagccacttggattgcagtggcctccctcctctctcagaccaatatccaagagaagagctcaccagaatagttcgcaatgcagatccaatagccaagtacttacaaaaagaaatgcaagtaattagaagtaatccttcatttaacatccccactgggtgcctcgaggtatttcctgaagccgaatggtcccagggtgttcagggaaccttacgaattaagaaatacttgactgtggagcaaataatgacctgtgtggcagacacgtgcaggcgcttctttgataggggctattctccaaaggatgttgctgtgcttgtcagcaccgcaaaagaagtggagcactataagtatgagctcttgaaagcaatgaggaagaaaagggtggtgcagctcagtgatgcatgtgatatgttgggtgatcacattgtgttggacagtgttcggcgattctcaggcctggaaaggagcatagtgtttgggatccatccaaggacagctgacccagctatcttacccaatgttctgatctgtctggcttccagggcaaaacaacacctgtatatttttccgtggggtggccattag